European Patent Application EP 4 549 565 A1, published May 7, 2025. Title: ｔｒａｃｒＲＮＡユニット、及びゲノム編集方法. Applicant: リージョナルフィッシュ株式会社. The sequence listing filed with the application follows.

SEQUENCE LISTING (17 sequences)

SEQ ID NO: 1 - RNA, 69 nt, Streptococcus pyogenes
  source 1..69: mol_type = other RNA
aaacagcatagcaagttaaaataaggctagtccgttatcaacttgaaaaagtggcaccgagtcggtgct

SEQ ID NO: 2 - RNA, 42 nt, synthetic construct
  misc_feature 1..42: note = crRNA
  misc_feature 1..20: note = n - n is a, g, t, or c
  source 1..42: mol_type = other RNA
nnnnnnnnnnnnnnnnnnnngttttagagctatgctgttttg

SEQ ID NO: 3 - DNA, 23 bp, Oryzias latipes
  source 1..23: mol_type = genomic DNA
acggagcgcactggaagctgagg

SEQ ID NO: 4 - RNA, 42 nt, synthetic construct
  misc_feature 1..42: note = tracr RNA fragment
  source 1..42: mol_type = other RNA
acggagcgcactggaagctggttttagagctatgctgttttg

SEQ ID NO: 5 - RNA, 61 nt, synthetic construct
  misc_feature 1..61: note = tracr RNA fragment
  source 1..61: mol_type = other RNA
tagcaagttaaaataaggctagtccgttatcaacttgaaaaagtggcaccgagtcggtgct

SEQ ID NO: 6 - RNA, 65 nt, synthetic construct
  misc_feature 1..65: note = tracr RNA fragment
  source 1..65: mol_type = other RNA
aaacagcatagcaagttaaaataaggctagtccgtaacttgaaaaagtggcaccgagtcggtgct

SEQ ID NO: 7 - RNA, 32 nt, synthetic construct
  misc_feature 1..32: note = tracr RNA fragment
  source 1..32: mol_type = other RNA
aaacagcatagcaagttaaaataaggctccgg

SEQ ID NO: 8 - RNA, 45 nt, synthetic construct
  misc_feature 1..45: note = tracr RNA fragment
  source 1..45: mol_type = other RNA
ccggagtccgttatcaacttgaaaaagtggcaccgagtcggtgct

SEQ ID NO: 9 - RNA, 48 nt, synthetic construct
  misc_feature 1..48: note = tracr RNA fragment
  source 1..48: mol_type = other RNA
aaacagcatagcaagttaaaataaggctagtccgttatcaacttggcc

SEQ ID NO: 10 - RNA, 25 nt, synthetic construct
  misc_feature 1..25: note = tracr RNA fragment
  source 1..25: mol_type = other RNA
ggccaagtggcaccgagtcggtgct

SEQ ID NO: 11 - RNA, 36 nt, synthetic construct
  misc_feature 1..36: note = tracr RNA fragment
  source 1..36: mol_type = other RNA
tagcaagttaaaataaggctagtccgtaacttggcc

SEQ ID NO: 12 - RNA, 24 nt, synthetic construct
  misc_feature 1..24: note = tracr RNA fragment
  source 1..24: mol_type = other RNA
ccggagtccgttatcaacttggcc

SEQ ID NO: 13 - RNA, 24 nt, synthetic construct
  misc_feature 1..24: note = tracr RNA fragment
  source 1..24: mol_type = other RNA
tagcaagttaaaataaggctccgg

SEQ ID NO: 14 - DNA, 25 bp, synthetic construct
  misc_feature 1..25: note = primer
  source 1..25: mol_type = other DNA
gtcactctgtattggggcgcctcct

SEQ ID NO: 15 - DNA, 25 bp, synthetic construct
  misc_feature 1..25: note = primer
  source 1..25: mol_type = other DNA
cttggcctgatctcagggctggatg

SEQ ID NO: 16-17 - skipped (2 entries)